European Patent Application EP 4 495 239 A1, published January 22, 2025. Title: Agents for treating cancer. Applicant: Ioannis Toumpoulis. Application EP. The sequence listing filed with the application follows.

SEQUENCE LISTING (146 sequences)

SEQ ID NO: 1 - RNA, 6229 nt, Homo sapiens
  source 1..6229: mol_type = mRNA
agacctctcctcattcttattgttttattagggcaatttgtctcaataaaagcccaggaagaagacgaggatgaaggatatggtgaagaaatagcctgcactcagaatggccagatgtacttaaacagggacatttggaaacctgccccttgtcagatctgtgtctgtgacaatggagccattctctgtgacaagatagaatgccaggatgtgctggactgtgccgaccctgtaacgccccctggggaatgctgtcctgtctgttcacaaacacctggaggtggcaataccaattttggtagaggaagaaagggacaaaagggagaaccaggattagtgcctgttgtaacaggcatacgtggtcgtccaggaccggcaggacctccaggatcacagggaccaagaggagagcgagggccaaaaggaagacctggccctcgtggacctcagggaattgatggagaaccaggtgttcctggtcaacctggtgctccaggacctcctggacatccgtcccacccaggacccgatggcttgagcaggccgttttcagctcaaatggctgggttggatgaaaaatctggacttgggagtcaagtaggactaatgcctggctctgtgggtcctgttggcccaaggggaccacagggtttacaaggacagcaaggtggtgcaggacctacaggacctcctggtgaacctggtgatcctggaccaatgggtccgattggttcacgtggaccagagggccctcctggtaaacctggggaagatggtgaacctggcagaaatggaaatcctggtgaagtgggatttgcaggatctccgggagctcgtggatttcctggggctcctggtcttccaggtctgaagggtcaccgaggacacaaaggtcttgaaggccctaaaggtgaagttggagcacctggttccaagggtgaagctggccccactggtccaatgggtgccatgggtcctctgggtccgaggggaatgccaggagagagagggagacttgggccacagggtgctcctggacaacgaggtgcacatggtatgcctggaaaacctggaccaatgggtcctcttgggataccaggctcttctggttttccaggaaatcctggaatgaagggagaagcaggtcctacaggggcgcgaggccctgaaggtcctcaggggcagagaggtgaaactgggcccccaggtccagttggctctccaggtcttcctggtgcaataggaactgatggtactcctggtgccaaaggcccaacgggctctccaggtacctctggtcctcctggctcagcagggcctcctggatctccaggacctcagggtagcactggtcctcagggaattcgaggccaaccgggtgatccaggagttccaggtttcaaaggagaagctggcccaaaaggggaaccagggccacatggtattcagggtccgataggcccacccggtgaagaaggcaaaagaggtcccagaggtgacccaggaacagttggtcctccagggccagtgggagaaaggggtgctcctggcaatcgtggttttccaggctctgatggtttacctgggccaaagggtgctcaaggagaacggggtcctgtaggttcttcaggacccaaaggaagccagggggatccaggacgtccaggggaacctgggcttccaggtgctcggggtttgacaggaaatcctggtgttcaaggtcctgaaggaaaacttggacctttgggtgcgccaggggaagatggccgtccaggtcctccaggctccataggaatcagagggcagcccgggagcatgggccttccaggccccaaaggtagcagtggtgaccctgggaaacctggagaagcaggaaatgctggagttcctgggcagaggggagctcctggaaaagatggtgaagttggtccttctggtcctgtgggcccgccgggtctagctggtgaaagaggagaacaaggacctccaggccccacaggttttcaggggcttcctggtcctccagggcctcctggagaaggtggaaaaccaggtgatcaaggtgttcctggagatcccggagcagttggcccgttaggacctagaggagaacgaggaaatcctggggaaagaggagaacctgggataactggactccctggtgagaagggaatggctggaggacatggtcctgatggcccaaaaggcagtccaggtccatctgggacccctggagatacaggcccaccaggtcttcaaggtatgccgggagaaagaggaattgcaggaactcctggccccaagggtgacagaggtggcataggagaaaaaggtgctgaaggcacagctggaaatgatggtgcaagaggtcttccaggtcctttgggccctccaggtccggcaggtcctactggagaaaagggtgaacctggtcctcgaggtttagttggccctcctggctcccggggcaatcctggttctcgaggtgaaaatgggccaactggagctgttggttttgccggaccccagggtcctgacggacagcctggagtaaaaggtgaacctggagagccaggacagaagggagatgctggttctcctggaccacaaggtttagcaggatcccctggccctcatggtcctaatggtgttcctggactaaaaggtggtcgaggaacccaaggtccgcctggtgctacaggatttcctggttctgcgggcagagttggacctccaggccctgctggagctccaggacctgcgggacccctaggggaacccgggaaggagggacctccaggtcttcgtggggaccctggctctcatgggcgtgtgggagatcgaggaccagctggcccccctggtggcccaggagacaaaggggacccaggagaagatgggcaacctggtccagatggcccccctggtccagctggaacgaccgggcagagaggaattgttggcatgcctgggcaacgtggagagagaggcatgcccggcctaccaggcccagcgggaacaccaggaaaagtaggaccaactggtgcaacaggagataaaggtccacctggacctgtggggcccccaggctccaatggtcctgtaggggaacctggaccagaaggtccagctggcaatgatggtaccccaggacgggatggtgctgttggagaacgtggtgatcgtggagaccctgggcctgcaggtctgccaggctctcagggtgcccctggaactcctggccctgtgggtgctccaggagatgcaggacaaagaggagatccgggttctcggggtcctataggaccacctggtcgagctgggaaacgtggattacctggaccccaaggacctcgtggtgacaaaggtgatcatggagaccgaggtgacagaggtcagaagggccacagaggctttactggtcttcagggtcttcctggccctcctggtccaaatggtgaacaaggaagtgctggaatccctggaccatttggcccaagaggtcctccaggcccagttggtccttcaggtaaagaaggaaaccctgggccacttgggccaattggacctccaggtgtacgaggcagtgtaggagaagcaggacctgagggccctcctggtgagcctggcccacctggccctccgggtccccctggccaccttacagctgctcttggggatatcatggggcactatgatgaaagcatgccagatccacttcctgagtttactgaagatcaggcggctcctgatgacaaaaacaaaacggacccaggggttcatgctaccctgaagtcactcagtagtcagattgaaaccatgcgcagccccgatggctcgaaaaagcacccagcccgcacgtgtgatgacctaaagctttgccattccgcaaagcagagtggtgaatactggattgatcctaaccaaggatctgttgaagatgcaatcaaagtttactgcaacatggaaacaggagaaacatgtatttcagcaaacccatccagtgtaccacgtaaaacctggtgggccagtaaatctcctgacaataaacctgtttggtatggtcttgatatgaacagagggtctcagttcgcttatggagaccaccaatcacctaatacagccattactcagatgacttttttgcgccttttatcaaaagaagcctcccagaacatcacttacatctgtaaaaacagtgtaggatacatggacgatcaagctaagaacctcaaaaaagctgtggttctcaaaggggcaaatgacttagatatcaaagcagagggaaatattagattccggtatatcgttcttcaagacacttgctctaagcggaatggaaatgtgggcaagactgtctttgaatatagaacacagaatgtggcacgcttgcccatcatagatcttgctcctgtggatgttggcggcacagaccaggaattcggcgttgaaattgggccagtttgttttgtgtaaagtaagccaagacacatcgacaatgagcaccaccatcaatgaccaccgccattcacaagaactttgactgtttgaagttgatcctgagactcttgaagtaatggctgatcctgcatcagcattgtatatatggtcttaagtgcctggcctccttatccttcagaatatttattttacttacaatcctcaagttttaattgattttaaatatttttcaatacaacagtttaggtttaagatgaccaatgacaatgaccacctttgcagaaagtaaactgattgaataaataaatctccgttttcttcaatttatttcagtgtaatgaaaaagttgcttagtatttatgaggaaattcttcttcctggcaggtagcttaaagagtggggtatatagagccacaacacatgtttattttgcttggctgcagttgaaaaatagaaattagtgcccttttgtgacctctcattccaagattgtcaattaaaaatgagtttaaaatgtttaacttgtgatcgagacctacatgcatgtcttgatattgtgtaactataatagagactctttaaggagaatcttaaaaaaaaaaaaacgtttctcactgtcttaaatagaatttttaaatagtatatattcagtggcattttggagaacaaagtgaatttacttcgacttcttaaatttttgtaaaagactataagtttagacatctttctcattcaaatttaaagatatctttctcctcttgatcaatctatcaatattgatagaagtcacactagtatataccatttaatacatttacactttcttatttaagaagatattgaatgcaaaataattgacatatagaactttacaaacatatgtccaaggactctaaattgagactcttccacatgtacaatctcatcatcctgaagcctataatgaagaaaaagatctagaaactgagttgtggagctgactctaatcaaatgtgatgattggaattagaccatttggcctttgaactttcataggaaaaatgacccaacatttcttagcatgagctacctcatctctagaagctgggatggacttactattcttgtttatattttagatactgaaaggtgctatgcttctgttattattccaagactggagataggcagggctaaaaaggtattattatttttcctttaatgatggtgctaaaattcttcctataaaattccttaaaaataaagatggtttaatcactaccattgtgaaaacataactgttagacttcccgtttctgaaagaaagagcatcgttccaatgcttgttcactgttcctctgtcatactgtatctggaatgctttgtaatacttgcatgcttcttagaccagaacatgtaggtccccttgtgtctcaatactttttttttcttaattgcatttgttggctctattttaatttttttcttttaaaataaacagctgggaccatcccaaaagacaagccatgcatacaactttggtcatgtatctctgcaaagcatcaaattaaatgcacgcttttgtcatgtcagtggtttttgttttgtgaaattcctttgaccatattagatctatttcatttccaatagtgaaaaggagatgtggtggtatactttgtttgccatttgtttaaaagatacaacggataccttctatcatgtatgtactggcttataaatgaaaatctatctacaacattacccacaaaggcaacatgacaccaattat

SEQ ID NO: 2 - RNA, 4773 nt, Homo sapiens
  source 1..4773: mol_type = mRNA
cacaattctccagagggaatatcaaaaacaacgggattttgcacaaacagaaagaattctaaaggctcagatactgcttacagagtttcaaagcaagcacaactcagtgccccaacaaaacagttatttccaggtggaactttcccagaagacttttcaatactatttacagtaaaaccaaaaaaaggaattcagtctttccttttatctatatataatgagcatggtattcagcaaattggtgttgaggttgggagatcacctgtttttctgtttgaagaccacactggaaaacctgccccagaagactatcccctcttcagaactgttaacatcgctgacgggaagtggcatcgggtagcaatcagcgtggagaagaaaactgtgacaatgattgttgattgtaagaagaaaaccacgaaaccacttgatagaagtgagagagcaattgttgataccaatggaatcacggtttttggaacaaggattttggatgaagaagtttttgagggggacattcagcagtttttgatcacaggtgatcccaaggcagcatatgactactgtgagcattatagtccagactgtgactcttcagcacccaaggctgctcaagctcaggaacctcagatagatgagtatgcaccagaggatataatcgaatatgactatgagtatggggaagcagagtataaagaggctgaaagtgtaacagagggacccactgtaactgaggagacaatagcacagacggaggcaaacatcgttgatgattttcaagaatacaactatggaacaatggaaagttaccagacagaagctcctaggcatgtttctgggacaaatgagccaaatccagttgaagaaatatttactgaagaatatctaacgggagaggattatgattcccagaggaaaaattctgaggatacactatatgaaaacaaagaaatagacggcagggattctgatcttctggtagatggagatttaggcgaatatgatttttatgaatataaagaatatgaagataaaccaacaagcccccctaatgaagaatttggtccaggtgtaccagcagaaactgatattacagaaacaagcataaatggccatggtgcatatggagagaaaggacagaaaggagaaccagcagtggttgagcctggtatgcttgtcgaaggaccaccaggaccagcaggacctgcaggtattatgggtcctccaggtctacaaggccccactggaccccctggtgaccctggcgataggggccccccaggacgtcctggcttaccaggggctgatggtctacctggtcctcctggtactatgttgatgttaccgttccgttatggtggtgatggttccaaaggaccaaccatctctgctcaggaagctcaggctcaagctattcttcagcaggctcggattgctctgagaggcccacctggcccaatgggtctaactggaagaccaggtcctgtgggggggcctggttcatctggggccaaaggtgagagtggtgatccaggtcctcagggccctcgaggcgtccagggtccccctggtccaacgggaaaacctggaaaaaggggtcgtccaggtgcagatggaggaagaggaatgccaggagaacctggggcaaagggagatcgagggtttgatggacttccgggtctgccaggtgacaaaggtcacaggggtgaacgaggtcctcaaggtcctccaggtcctcctggtgatgatggaatgaggggagaagatggagaaattggaccaagaggtcttccaggtgaagctggcccacgaggtttgctgggtccaaggggaactccaggagctccagggcagcctggtatggcaggtgtagatggccccccaggaccaaaagggaacatgggtccccaaggggagcctgggcctccaggtcaacaagggaatccaggacctcagggtcttcctggtccacaaggtccaattggtcctcctggtgaaaaaggaccacaaggaaaaccaggacttgctggacttcctggtgctgatgggcctcctggtcatcctgggaaagaaggccagtctggagaaaagggggctctgggtccccctggtccacaaggtcctattggatacccgggcccccggggagtaaagggagcagatggtgtcagaggtctcaagggatctaaaggtgaaaagggtgaagatggttttccaggattcaaaggtgacatgggtctaaaaggtgacagaggagaagttggtcaaattggcccaagaggggaagatggccctgaaggacccaaaggtcgagcaggcccaactggagacccaggtccttcaggtcaagcaggagaaaagggaaaacttggagttccaggattaccaggatatccaggaagacaaggtccaaagggttccactggattccctgggtttccaggtgccaatggagagaaaggtgcacggggagtagctggcaaaccaggccctcggggtcagcgtggtccaacgggtcctcgaggttcaagaggtgcaagaggtcccactgggaaacctgggccaaagggcacttcaggtggcgatggccctcctggccctccaggtgaaagaggtcctcaaggacctcagggtccagttggattccctggaccaaaaggccctcctggaccacctgggaaggatgggctgccaggacaccctgggcaacgtggggagactggatttcaaggcaagaccggccctcctgggccagggggagtggttggaccacagggaccaaccggtgagactggtccaataggggaacgtgggcatcctggccctcctggccctcctggtgagcaaggtcttcctggtgctgcaggaaaagaaggtgcaaagggtgatccaggtcctcaaggtatctcagggaaagatggaccagcaggattacgtggtttcccaggggaaagaggtcttcctggagctcagggtgcacctggactgaaaggaggggaaggtccccagggcccaccaggtccagttggctcaccaggagaacgtgggtcagcaggtacagctggcccaattggtttaccagggcgcccgggacctcagggtcctcctggtccagctggagagaaaggtgctcctggagaaaaaggtccccaagggcctgcagggagagatggagttcaaggtcctgttggtctcccagggccagctggtcctgccggctcccctggggaagacggagacaagggtgaaattggtgagccgggacaaaaaggcagcaagggtgacaagggagaaaatggccctcccggtcccccaggtcttcaaggaccagttggtgcccctggaattgctggaggtgatggtgaaccaggtcctagaggacagcaggggatgtttgggcaaaaaggtgatgagggtgccagaggcttccctggacctcctggtccaataggtcttcagggtctgccaggcccacctggtgaaaaaggtgaaaatggggatgttggtcccatggggccacctggtcctccaggcccaagaggccctcaaggtcccaatggagctgatggaccacaaggacccccagggtctgttggttcagttggtggtgttggagaaaagggtgaacctggagaagcagggaacccagggcctcctggggaagcaggtgtaggcggtcccaaaggagaaagaggagagaaaggggaagctggtccacctggagctgctggacctccaggtgccaaggggccaccaggtgatgatggccctaagggtaacccgggtcctgttggttttcctggagatcctggtcctcctggggaacctggccctgcaggtcaagatggtgttggtggtgacaagggtgaagatggagatcctggtcaaccgggtcctcctggcccatctggtgaggctggcccaccaggtcctcctggaaaacgaggtcctcctggagctgcaggtgcagagggaagacaaggtgaaaaaggtgctaagggggaagcaggtgcagaaggtcctcctggaaaaaccggcccagtcggtcctcagggacctgcaggaaagcctggtccagaaggtcttcggggcatccctggtcctgtgggagaacaaggtctccctggagctgcaggccaagatggaccacctggtcctatgggacctcctggcttacctggtctcaaaggtgaccctggctccaagggtgaaaagggacatcctggtttaattggcctgattggtcctccaggagaacaaggggaaaaaggtgaccgagggctccctggaactcaaggatctccaggagcaaaaggggatgggggaattcctggtcctgctggtcccttaggtccacctggtcctccaggtttaccaggtcctcaaggcccaaagggtaacaaaggctctactggacccgctggccagaaaggtgacagtggtcttccagggcctcctgggtctccaggtccacctggtgaagtcattcagcctttaccaatcttgtcctccaaaaaaacgagaagacatactgaaggcatgcaagcagatgcagatgataatattcttgattactcggatggaatggaagaaatatttggttccctcaattccctgaaacaagacattgagcatatgaaatttccaatgggtactcagaccaatccagcccgaacttgtaaagacctgcaactcagccatcctgacttcccagatggtgaatattggattgatcctaaccaaggttgctcaggagattccttcaaagtttac

SEQ ID NO: 3 - RNA, 1867 nt, Homo sapiens
  source 1..1867: mol_type = mRNA
catcacctattggatccaaaactactcggaagacttgccgcgggcggtgattgacgacgcctttgcccgcgccttcgcactgtggagcgcggtgacgccgctcaccttcactcgcgtgtacagccgggacgcagacatcgtcatccagtttggtgtcgcggagcacggagacgggtatcccttcgacgggaaggacgggctcctggcacacgcctttcctcctggccccggcattcagggagacgcccatttcgacgatgacgagttgtggtccctgggcaagggcgtcgtggttccaactcggtttggaaacgcagatggcgcggcctgccacttccccttcatcttcgagggccgctcctactctgcctgcaccaccgacggtcgctccgacggcttgccctggtgcagtaccacggccaactacgacaccgacgaccggtttggcttctgccccagcgagagactctacacccaggacggcaatgctgatgggaaaccctgccagtttccattcatcttccaaggccaatcctactccgcctgcaccacggacggtcgctccgacggctaccgctggtgcgccaccaccgccaactacgaccgggacaagctcttcggcttctgcccgacccgagctgactcgacggtgatggggggcaactcggcgggggagctgtgcgtcttccccttcactttcctgggtaaggagtactcgacctgtaccagcgagggccgcggagatgggcgcctctggtgcgctaccacctcgaactttgacagcgacaagaagtggggcttctgcccggaccaaggatacagtttgttcctcgtggcggcgcatgagttcggccacgcgctgggcttagatcattcctcagtgccggaggcgctcatgtaccctatgtaccgcttcactgaggggccccccttgcataaggacgacgtgaatggcatccggcacctctatggtcctcgccctgaacctgagccacggcctccaaccaccaccacaccgcagcccacggctcccccgacggtctgccccaccggaccccccactgtccacccctcagagcgccccacagctggccccacaggtcccccctcagctggccccacaggtccccccactgctggcccttctacggccactactgtgcctttgagtccggtggacgatgcctgcaacgtgaacatcttcgacgccatcgcggagattgggaaccagctgtatttgttcaaggatgggaagtactggcgattctctgagggcagggggagccggccgcagggccccttccttatcgccgacaagtggcccgcgctgccccgcaagctggactcggtctttgaggagcggctctccaagaagcttttcttcttctctgggcgccaggtgtgggtgtacacaggcgcgtcggtgctgggcccgaggcgtctggacaagctgggcctgggagccgacgtggcccaggtgaccggggccctccggagtggcagggggaagatgctgctgttcagcgggcggcgcctctggaggttcgacgtgaaggcgcagatggtggatccccggagcgccagcgaggtggaccggatgttccccggggtgcctttggacacgcacgacgtcttccagtaccgagagaaagcctatttctgccaggaccgcttctactggcgcgtgagttcccggagtgagttgaaccaggtggaccaagtgggctacgtgacctatgacatcctgcagtgccctgaggactagggctcccgtcctgctttggcagtgccatgtaaatccccactgggaccaaccctggggaaggagccagtttgccggatacaaactggtattctgttctggagg

SEQ ID NO: 4 - RNA, 2743 nt, Homo sapiens
  source 1..2743: mol_type = mRNA
atcatgtggagaatgtatacaagcagggccaaattgtgggtggtgcacaaattcaacatttttacaggaaggaatgcctacttctgcacgatgtgatgatttagaagccttaaaaaagaagggttgccctccagatgacatagaaaatcccagaggctccaaagatataaagaaaaataaaaatgtaaccaaccgtagcaaaggaacagcagagaagctcaagccagaggatattactcagatccaaccacagcagttggttttgcgattaagatcaggggagccacagacatttacattaaaattcaagagagctgaagactatcccattgacctctactaccttatggacctgtcttactcaatgaaagacgatttggagaatgtaaaaagtcttggaacagatctgatgaatgaaatgaggaggattacttcggacttcagaattggatttggctcatttgtggaaaagactgtgatgccttacattagcacaacaccagctaagctcaggaacccttgcacaagtgaacagaactgcaccagcccatttagctacaaaaatgtgctcagtcttactaataaaggagaagtatttaatgaacttgttggaaaacagcgcatatctggaaatttggattctccagaaggtggtttcgatgccatcatgcaagttgcagtttgtggatcactgattggctggaggaatgttacacggctgctggtgttttccacagatgccgggtttcactttgctggagatgggaaacttggtggcattgttttaccaaatgatggacaatgtcacctggaaaataatatgtacacaatgagccattattatgattatccttctattgctcaccttgtccagaaactgagtgaaaataatattcagacaatttttgcagttactgaagaatttcagcctgtttacaaggagctgaaaaacttgatccctaagtcagcagtaggaacattatctgcaaattctagcaatgtaattcagttgatcattgatgcatacaattccctttcctcagaagtcattttggaaaacggcaaattgtcagaaggcgtaacaataagttacaaatcttactgcaagaacggggtgaatggaacaggggaaaatggaagaaaatgttccaatatttccattggagatgaggttcaatttgaaattagcataacttcaaataagtgtccaaaaaaggattctgacagctttaaaattaggcctctgggctttacggaggaagtagaggttattcttcagtacatctgtgaatgtgaatgccaaagcgaaggcatccctgaaagtcccaagtgtcatgaaggaaatgggacatttgagtgtggcgcgtgcaggtgcaatgaagggcgtgttggtagacattgtgaatgcagcacagatgaagttaacagtgaagacatggatgcttactgcaggaaagaaaacagttcagaaatctgcagtaacaatggagagtgcgtctgcggacagtgtgtttgtaggaagagggataatacaaatgaaatttattctggcaaattctgcgagtgtgataatttcaactgtgatagatccaatggcttaatttgtggaggaaatggtgtttgcaagtgtcgtgtgtgtgagtgcaaccccaactacactggcagtgcatgtgactgttctttggatactagtacttgtgaagccagcaacggacagatctgcaatggccggggcatctgcgagtgtggtgtctgtaagtgtacagatccgaagtttcaagggcaaacgtgtgagatgtgtcagacctgccttggtgtctgtgctgagcataaagaatgtgttcagtgcagagccttcaataaaggagaaaagaaagacacatgcacacaggaatgttcctattttaacattaccaaggtagaaagtcgggacaaattaccccagccggtccaacctgatcctgtgtcccattgtaaggagaaggatgttgacgactgttggttctattttacgtattcagtgaatgggaacaacgaggtcatggttcatgttgtggagaatccagagtgtcccactggtccagacatcattccaattgtagctggtgtggttgctggaattgttcttattggccttgcattactgctgatatggaagcttttaatgataattcatgacagaagggagtttgctaaatttgaaaaggagaaaatgaatgccaaatgggacacgggtgaaaatcctatttataagagtgccgtaacaactgtggtcaatccgaagtatgagggaaaatgagtactgcccgtgcaaatcccacaacactgaatgcaaagtagcaatttccatagtcacagttaggtagctttagggcaatattgccatggttttactcatgtgcaggttttgaaaatgtacaatatgtataatttttaaaatgttttattattttgaaaataatgttgtaattcatgccagggactgacaaaagacttgagacaggatggttactcttgtcagctaaggtcacattgtgcctttttgaccttttcttcctggactattgaaatcaagcttattggattaagtgatatttctatagcgattgaaagggcaatagttaaagtaatgagcatgatgagagtttctgttaatcatgtattaaaactgatttttagctttacaaatatgtcagtttgcagttatgcagaatccaaagtaaatgtcctgctagctagttaa

SEQ ID NO: 5 - RNA, 1832 nt, Homo sapiens
  source 1..1832: mol_type = mRNA
cgaggacagctatattgtgttcacctatcgaccttgcgggtgctgctcctacgtgggtcgccgcggcgggggcccccaggccatctccatcggcaagaactgtgacaagttcggcattgtggtccacgagctgggccacgtcgtcggcttctggcacgaacacactcggccagaccgggaccgccacgtttccatcgttcgtgagaacatccagccagggcaggagtataacttcctgaagatggagcctcaggaggtggagtccctgggggagacctatgacttcgacagcatcatgcattacgctcggaacacattctccaggggcatcttcctggataccattgtccccaagtatgaggtgaacggggtgaaacctcccattggccaaaggacacggctcagcaagggggacattgcccaagcccgcaagctttacaagtgcccagcctgtggagagaccctgcaagacagcacaggcaacttctcctcccctgaataccccaatggctactctgctcacatgcactgcgtgtggcgcatctctgtcacacccggggagaagatcatcctgaacttcacgtccctggacctgtaccgcagccgcctgtgctggtacgactatgtggaggtccgagatggcttctggaggaaggcgcccctccgaggccgcttctgcgggtccaaactccctgagcctatcgtctccactgacagccgcctctgggttgaattccgcagcagcagcaattgggttggaaagggcttctttgcagtctacgaagccatctgcgggggtgatgtgaaaaaggactatggccacattcaatcgcccaactacccagacgattaccggcccagcaaagtctgcatctggcggatccaggtgtctgagggcttccacgtgggcctcacattccagtcctttgagattgagcgccacgacagctgtgcctacgactatctggaggtgcgcgacgggcacagtgagagcagcaccctcatcgggcgctactgtggctatgagaagcctgatgacatcaagagcacgtccagccgcctctggctcaagttcgtctctgacgggtccattaacaaagcgggctttgccgtcaactttttcaaagaggtggacgagtgctctcggcccaaccgcgggggctgtgagcagcggtgcctcaacaccctgggcagctacaagtgcagctgtgaccccgggtacgagctggccccagacaagcgccgctgtgaggctgcttgtggcggattcctcaccaagctcaacggctccatcaccagcccgggctggcccaaggagtacccccccaacaagaactgcatctggcagctggtggcccccacccagtaccgcatctccctgcagtttgacttctttgagacagagggcaatgatgtgtgcaagtacgacttcgtggaggtgcgcagtggactcacagctgactccaagctgcatggcaagttctgtggttctgagaagcccgaggtcatcacctcccagtacaacaacatgcgcgtggagttcaagtccgacaacaccgtgtccaaaaagggcttcaaggcccacttcttctcagaaaagaggccagctctgcagccccctcggggacgcccccaccagctcaaattccgagtgcagaaaagaaaccggaccccccagtgaggcctgccaggcctcccggaccccttgttactcaggaacctcaccttggacggaatgggatgggggcttcggtgcccaccaaccccccacctccactctgccattccggcccacctccctctggccggacagaactggtgctctcttctcc

SEQ ID NO: 6 - RNA, 1339 nt, Homo sapiens
  source 1..1339: mol_type = mRNA
tctatgacaagttcaagcagagtacacacagcatatatatgttcttcaacacatcagagctccgagaagcggtacctgaacccgtgttgctctcccgggcagagctgcgtctgctgaggctcaagttaaaagtggagcagcacgtggagctgtaccagaaatacagcaacaattcctggcgatacctcagcaaccggctgctggcacccagcgactcgccagagtggttatcttttgatgtcaccggagttgtgcggcagtggttgagccgtggaggggaaattgagggctttcgccttagcgcccactgctcctgtgacagcagggataacacactgcaagtggacatcaacgggttcactaccggccgccgaggtgacctggccaccattcatggcatgaaccggcctttcctgcttctcatggccaccccgctggagagggcccagcatctgcaaagctcccggcaccgccgagccctggacaccaactattgcttcagctccacggagaagaactgctgcgtgcggcagctgtacattgacttccgcaaggacctcggctggaagtggatccacgagcccaagggctaccatgccaacttctgcctcgggccctgcccctacatttggagcctggacacgcagtacagcaaggtcctggccctgtacaaccagcataacccgggcgcctcggcggcgccgtgctgcgtgccgcaggcgctggagccgctgcccatcgtgtactacgtgggccgcaagcccaaggtggagcagctgtccaacatgatcgtgcgctcctgcaagtgcagctgaggtcccgccccgccccgccccgccccggcaggcccggccccaccccgccccgcccccgctgccttgcccatgggggctgtatttaaggacacccgtgccccaagcccacctggggccccattaaagatggagagaggactgcggatctctgtgtcattgggcgcctgcctggggtctccatccctgacgttcccccactcccactccctctctctccctctctgcctcctcctgcctgtctgcactattcctttgcccggcatcaaggcacaggggaccagtggggaacactactgtagttagatctatttattgagcaccttgggcactgttgaagtgccttacattaatgaactcattcagtcaccatagcaacactctgagatgcagggactctgataacacccattttaaaggtgaggaaacaagcccagagaggttaagggaggagttcctgcccaccaggaacctgctttagtgggggatagtgaagaagacaataaaagatagtagttcaggccagg

SEQ ID NO: 7 - protein, 4 aa, Homo sapiens
KGRR

SEQ ID NO: 8 - protein, 5 aa, Homo sapiens
KPGRR

SEQ ID NO: 9 - protein, 7 aa, Homo sapiens
GRSKRKK

SEQ ID NO: 10 - protein, 7 aa, Homo sapiens
RTWKKRK

SEQ ID NO: 11 - protein, 8 aa, Homo sapiens
GHRGGVVP

SEQ ID NO: 12 - protein, 5 aa, Homo sapiens
KGRRR

SEQ ID NO: 13 - protein, 9 aa, Homo sapiens
NNIRRRQNR

SEQ ID NO: 14 - protein, 5 aa, Homo sapiens
RGRKG

SEQ ID NO: 15 - protein, 4 aa, Homo sapiens
RGRK

SEQ ID NO: 16 - protein, 12 aa, Homo sapiens
SPDNKVQKKRVV

SEQ ID NO: 17 - protein, 17 aa, Homo sapiens
WSKSPDNKVKRVDVGTQ

SEQ ID NO: 18 - protein, 4 aa, Homo sapiens
KKRR

SEQ ID NO: 19 - protein, 7 aa, Homo sapiens
RWKTKRW

SEQ ID NO: 20 - protein, 6 aa, Homo sapiens
SKKTRR

SEQ ID NO: 21 - protein, 8 aa, Homo sapiens
LLFRYQRL

SEQ ID NO: 22 - protein, 5 aa, Homo sapiens
KKRGR

SEQ ID NO: 23 - protein, 4 aa, Homo sapiens
RRRR

SEQ ID NO: 24 - protein, 7 aa, Homo sapiens
RNRRRAY

SEQ ID NO: 25 - protein, 14 aa, Homo sapiens
RLTARRRRRGLRAY

SEQ ID NO: 26 - protein, 11 aa, Homo sapiens
SEEEKQKRKMK

SEQ ID NO: 27 - protein, 15 aa, Homo sapiens
SNQKTKGRFKHHQRK

SEQ ID NO: 28 - skipped

SEQ ID NO: 29 - protein, 4 aa, Homo sapiens
GRRT

SEQ ID NO: 30 - protein, 5 aa, Homo sapiens
PGRRR

SEQ ID NO: 31 - protein, 11 aa, Homo sapiens
SQKQKGRKHRK

SEQ ID NO: 32 - protein, 7 aa, Homo sapiens
RKKKSKT

SEQ ID NO: 33 - protein, 11 aa, Homo sapiens
DRSRRRVNSLP

SEQ ID NO: 34 - protein, 8 aa, Homo sapiens
REKRKKKT

SEQ ID NO: 35 - protein, 8 aa, Homo sapiens
RGKKKSKT

SEQ ID NO: 36 - protein, 10 aa, Homo sapiens
RKLKRDRNKR

SEQ ID NO: 37 - protein, 10 aa, Homo sapiens
RKKRSDRNKR

SEQ ID NO: 38 - protein, 13 aa, Homo sapiens
NSAAKKKRTNEYS

SEQ ID NO: 39 - protein, 14 aa, Homo sapiens
RSKGTKKRSDRNKR

SEQ ID NO: 40 - protein, 14 aa, Homo sapiens
NKGTSGRVQCVCKK

SEQ ID NO: 41 - protein, 18 aa, Homo sapiens
NQGPSAAKKCKRTNEYGN

SEQ ID NO: 42 - protein, 10 aa, Homo sapiens
PKRNSNTSKR

SEQ ID NO: 43 - protein, 13 aa, Homo sapiens
WKNKKYRNKKMDP

SEQ ID NO: 44 - protein, 8 aa, Homo sapiens
NKKYRNKK

SEQ ID NO: 45 - protein, 10 aa, Homo sapiens
KNKYRNEVKK

SEQ ID NO: 46 - protein, 12 aa, Homo sapiens
YRRVARRKKMVR

SEQ ID NO: 47 - protein, 14 aa, Homo sapiens
RVAKQRDKGLGAWR

SEQ ID NO: 48 - protein, 6 aa, Homo sapiens
RSRKRK

SEQ ID NO: 49 - protein, 6 aa, Homo sapiens
RKRDRR

SEQ ID NO: 50 - protein, 6 aa, Homo sapiens
RRRKRK

SEQ ID NO: 51 - protein, 11 aa, Homo sapiens
YRVAYRKGGRW

SEQ ID NO: 52 - protein, 13 aa, Homo sapiens
YRVARRKGADRWP

SEQ ID NO: 53 - protein, 8 aa, Homo sapiens
RRRSTKNW

SEQ ID NO: 54 - protein, 7 aa, Homo sapiens
RRRTKNW

SEQ ID NO: 55 - protein, 11 aa, Homo sapiens
RRRTKNPYIWQ

SEQ ID NO: 56 - protein, 10 aa, Homo sapiens
TKKGTTRAHR

SEQ ID NO: 57 - protein, 14 aa, Homo sapiens
THKKDGTTGRLAHR

SEQ ID NO: 58 - protein, 11 aa, Homo sapiens
TFKQSGFTTRR

SEQ ID NO: 59 - protein, 14 aa, Homo sapiens
ETHFKSIYGFTGRR

SEQ ID NO: 60 - protein, 6 aa, Homo sapiens
RGRPRK

SEQ ID NO: 61 - protein, 8 aa, Homo sapiens
GRSRSRRR

SEQ ID NO: 62 - protein, 6 aa, Homo sapiens
RGRSRR

SEQ ID NO: 63 - protein, 14 aa, Homo sapiens
SRSRRRDDRHKEYK

SEQ ID NO: 64 - protein, 10 aa, Homo sapiens
RSRRRKQSLG

SEQ ID NO: 65 - protein, 12 aa, Homo sapiens
QRSRPDRRRFKE

SEQ ID NO: 66 - protein, 12 aa, Homo sapiens
SRSRRRPRKYKY

SEQ ID NO: 67 - RNA, 19 nt, synthetic construct
  source 1..19: mol_type = other RNA
agacctctcctcattctta

SEQ ID NO: 68 - RNA, 19 nt, synthetic construct
  source 1..19: mol_type = other RNA
acacctggaggtggcaata

SEQ ID NO: 69 - RNA, 19 nt, synthetic construct
  source 1..19: mol_type = other RNA
tcctggttctcgaggtgaa

SEQ ID NO: 70 - RNA, 19 nt, Synthetic construct
  source 1..19: mol_type = other RNA
acaaggaagtgctggaatc

SEQ ID NO: 71 - RNA, 19 nt, synthetic construct
  source 1..19: mol_type = other RNA
atactggattgatcctaac

SEQ ID NO: 72 - RNA, 19 nt, synthetic construct
  source 1..19: mol_type = other RNA
tgagcaccaccatcaatga

SEQ ID NO: 73 - RNA, 19 nt, synthetic construct
  source 1..19: mol_type = other RNA
tgtgatgattggaattaga

SEQ ID NO: 74 - RNA, 19 nt, synthetic construct
  source 1..19: mol_type = other RNA
agacaagccatgcatacaa

SEQ ID NO: 75 - RNA, 19 nt, synthetic construct
  source 1..19: mol_type = other RNA
aaggagatgtggtggtata

SEQ ID NO: 76 - RNA, 19 nt, synthetic construct
  source 1..19: mol_type = other RNA
ggcaacatgacaccaatta

SEQ ID NO: 77 - RNA, 25 nt, synthetic construct
  source 1..25: mol_type = other RNA
cacaattctccagagggaatatcaa

SEQ ID NO: 78 - RNA, 25 nt, synthetic construct
  source 1..25: mol_type = other RNA
tgatagaagtgagagagcaattgtt

SEQ ID NO: 79 - RNA, 25 nt, synthetic construct
  source 1..25: mol_type = other RNA
cattatagtccagactgtgactctt

SEQ ID NO: 80 - RNA, 25 nt, synthetic construct
  source 1..25: mol_type = other RNA
agagtataaagaggctgaaagtgta

SEQ ID NO: 81 - RNA, 25 nt, synthetic construct
  source 1..25: mol_type = other RNA
cggaggcaaacatcgttgatgattt

SEQ ID NO: 82 - RNA, 25 nt, synthetic construct
  source 1..25: mol_type = other RNA
gatggagatttaggcgaatatgatt

SEQ ID NO: 83 - RNA, 25 nt, synthetic construct
  source 1..25: mol_type = other RNA
catcctggtttaattggcctgattg

SEQ ID NO: 84 - RNA, 25 nt, synthetic construct
  source 1..25: mol_type = other RNA
cagcctttaccaatcttgtcctcca

SEQ ID NO: 85 - RNA, 25 nt, synthetic construct
  source 1..25: mol_type = other RNA
cagaccaatccagcccgaacttgta

SEQ ID NO: 86 - RNA, 25 nt, synthetic construct
  source 1..25: mol_type = other RNA
gctcaggagattccttcaaagttta

SEQ ID NO: 87 - RNA, 19 nt, synthetic construct
  source 1..19: mol_type = other RNA
catcacctattggatccaa

SEQ ID NO: 88 - RNA, 19 nt, synthetic construct
  source 1..19: mol_type = other RNA
actactcggaagacttgcc

SEQ ID NO: 89 - RNA, 19 nt, synthetic construct
  source 1..19: mol_type = other RNA
aggagtactcgacctgtac

SEQ ID NO: 90 - RNA, 19 nt, synthetic construct
  source 1..19: mol_type = other RNA
tgcctgcaacgtgaacatc

SEQ ID NO: 91 - RNA, 19 nt, synthetic construct
  source 1..19: mol_type = other RNA
acgtgaacatcttcgacgc

SEQ ID NO: 92 - RNA, 19 nt, synthetic construct
  source 1..19: mol_type = other RNA
gtactggcgattctctgag

SEQ ID NO: 93 - RNA, 19 nt, synthetic construct
  source 1..19: mol_type = other RNA
actggtattctgttctgga

SEQ ID NO: 94 - RNA, 19 nt, synthetic construct
  source 1..19: mol_type = other RNA
ctggtattctgttctggag

SEQ ID NO: 95 - RNA, 19 nt, synthetic construct
  source 1..19: mol_type = other RNA
atcatgtggagaatgtata

SEQ ID NO: 96 - RNA, 19 nt, synthetic construct
  source 1..19: mol_type = other RNA
tcatgtggagaatgtatac

SEQ ID NO: 97 - RNA, 19 nt, synthetic construct
  source 1..19: mol_type = other RNA
aagactgtgatgccttaca

SEQ ID NO: 98 - RNA, 19 nt, synthetic construct
  source 1..19: mol_type = other RNA
aatgtgctcagtcttacta

SEQ ID NO: 99 - RNA, 19 nt, synthetic construct
  source 1..19: mol_type = other RNA
atgtgctcagtcttactaa

SEQ ID NO: 100 - RNA, 19 nt, synthetic construct
  source 1..19: mol_type = other RNA
tgtacacaatgagccatta

SEQ ID NO: 101 - RNA, 19 nt, synthetic construct
  source 1..19: mol_type = other RNA
caatgagccattattatga

SEQ ID NO: 102 - RNA, 19 nt, synthetic construct
  source 1..19: mol_type = other RNA
gtcagcagtaggaacatta

SEQ ID NO: 103 - RNA, 19 nt, synthetic construct
  source 1..19: mol_type = other RNA
attgtcagaaggcgtaaca

SEQ ID NO: 104 - RNA, 19 nt, synthetic construct
  source 1..19: mol_type = other RNA
atgtcctgctagctagtta

SEQ ID NO: 105 - RNA, 19 nt, synthetic construct
  source 1..19: mol_type = other RNA
tctatgacaagttcaagca

SEQ ID NO: 106 - RNA, 19 nt, synthetic construct
  source 1..19: mol_type = other RNA
gcagagtacacacagcata

SEQ ID NO: 107 - RNA, 19 nt, synthetic construct
  source 1..19: mol_type = other RNA
cacatcagagctccgagaa

SEQ ID NO: 108 - RNA, 19 nt, synthetic construct
  source 1..19: mol_type = other RNA
cacactgcaagtggacatc

SEQ ID NO: 109 - RNA, 19 nt, synthetic construct
  source 1..19: mol_type = other RNA
gcagctgtccaacatgatc

SEQ ID NO: 110 - RNA, 19 nt, synthetic construct
  source 1..19: mol_type = other RNA
acactactgtagttagatc

SEQ ID NO: 111 - RNA, 19 nt, synthetic construct
  source 1..19: mol_type = other RNA
gtgccttacattaatgaac

SEQ ID NO: 112 - RNA, 19 nt, synthetic construct
  source 1..19: mol_type = other RNA
tgaactcattcagtcacca

SEQ ID NO: 113 - RNA, 19 nt, synthetic construct
  source 1..19: mol_type = other RNA
ctcattcagtcaccatagc

SEQ ID NO: 114 - RNA, 19 nt, synthetic construct
  source 1..19: mol_type = other RNA
agatagtagttcaggccag

SEQ ID NO: 115 - RNA, 19 nt, synthetic construct
  source 1..19: mol_type = other RNA
cgaggacagctatattgtg

SEQ ID NO: 116 - RNA, 19 nt, synthetic construct
  source 1..19: mol_type = other RNA
ggacagctatattgtgttc

SEQ ID NO: 117 - RNA, 19 nt, synthetic construct
  source 1..19: mol_type = other RNA
agacagcacaggcaacttc

SEQ ID NO: 118 - RNA, 19 nt, synthetic construct
  source 1..19: mol_type = other RNA
tggctactctgctcacatg

SEQ ID NO: 119 - RNA, 19 nt, synthetic construct
  source 1..19: mol_type = other RNA
gaagatcatcctgaacttc

SEQ ID NO: 120 - RNA, 19 nt, synthetic construct
  source 1..19: mol_type = other RNA
agatcatcctgaacttcac

SEQ ID NO: 121 - RNA, 19 nt, synthetic construct
  source 1..19: mol_type = other RNA
aggactatggccacattca

SEQ ID NO: 122 - RNA, 19 nt, synthetic construct
  source 1..19: mol_type = other RNA
ggactatggccacattcaa

SEQ ID NO: 123 - RNA, 19 nt, synthetic construct
  source 1..19: mol_type = other RNA
gttctgtggttctgagaag

SEQ ID NO: 124 - RNA, 19 nt, synthetic construct
  source 1..19: mol_type = other RNA
gaactggtgctctcttctc

SEQ ID NO: 125 - RNA, 19 nt, synthetic construct
  source 1..19: mol_type = other RNA
agacctctcctcattctta

SEQ ID NO: 126 - RNA, 25 nt, synthetic construct
  source 1..25: mol_type = other RNA
gctcaggagattccttcaaagttta

SEQ ID NO: 127 - RNA, 19 nt, synthetic construct
  source 1..19: mol_type = other RNA
catcacctattggatccaa

SEQ ID NO: 128 - RNA, 19 nt, synthetic construct
  source 1..19: mol_type = other RNA
gtcagcagtaggaacatta

SEQ ID NO: 129 - RNA, 19 nt, synthetic construct
  source 1..19: mol_type = other RNA
ggactatggccacattcaa

SEQ ID NO: 130 - RNA, 19 nt, synthetic construct
  source 1..19: mol_type = other RNA
gcagagtacacacagcata

SEQ ID NO: 131 - RNA, 19 nt, synthetic construct
  source 1..19: mol_type = other RNA
gcctatcttacactcctat

SEQ ID NO: 132 - RNA, 25 nt, synthetic construct
  source 1..25: mol_type = other RNA
gcgtcttaaggaactagtctattca

SEQ ID NO: 133 - DNA, 21 bp, synthetic construct
  source 1..21: mol_type = other DNA
ggcttccttcgttattggagc

SEQ ID NO: 134 - DNA, 20 bp, synthetic construct
  source 1..20: mol_type = other DNA
accgatcaaccgttcagtgt

SEQ ID NO: 135 - DNA, 22 bp, synthetic construct
  source 1..22: mol_type = other DNA
actgcaacatggaaacaggaga

SEQ ID NO: 136 - DNA, 21 bp, synthetic construct
  source 1..21: mol_type = other DNA
gattggtggtctccataagcg

SEQ ID NO: 137 - DNA, 21 bp, synthetic construct
  source 1..21: mol_type = other DNA
acactgtatgatggttgtgcg

SEQ ID NO: 138 - DNA, 22 bp, synthetic construct
  source 1..22: mol_type = other DNA
acaggaccaacttcaaatccga

SEQ ID NO: 139 - DNA, 20 bp, synthetic construct
  source 1..20: mol_type = other DNA
aagcgaaggcatccctgaaa

SEQ ID NO: 140 - DNA, 20 bp, synthetic construct
  source 1..20: mol_type = other DNA
gcagacgcactctccattgt

SEQ ID NO: 141 - DNA, 19 bp, synthetic construct
  source 1..19: mol_type = other DNA
cctctggaggttcgacgtg

SEQ ID NO: 142 - DNA, 20 bp, synthetic construct
  source 1..20: mol_type = other DNA
aactcacgcgccagtagaag

SEQ ID NO: 143 - DNA, 21 bp, synthetic construct
  source 1..21: mol_type = other DNA
gcaacaattcctggcgatacc

SEQ ID NO: 144 - DNA, 21 bp, synthetic construct
  source 1..21: mol_type = other DNA
tagtgaacccgttgatgtcca

SEQ ID NO: 145 - DNA, 20 bp, synthetic construct
  source 1..20: mol_type = other DNA
gcctgtgctggtacgactat

SEQ ID NO: 146 - DNA, 20 bp, synthetic construct
  source 1..20: mol_type = other DNA
cgcagatggcttcgtagact